European Patent Specification EP 3 313 891 B1, published April 1, 2026. Title: FACTOR XI ANTIBODIES AND METHODS OF USE. Applicant: NOVARTIS AG. The sequence listing filed with the application follows.

SEQUENCE LISTING (51 sequences)

SEQ ID NO: 1 - protein, 625 aa, Homo sapiens [sequence omitted]

SEQ ID NO: 2 - DNA, 3278 bp, Homo sapiens
aggcacacaggcaaaatcaagttctacatctgtccctgtgtatgtcacttgtttgaatacgaaataaaattaaaaaaataaattcagtgtattgagaaagcaagcaattctctcaaggtatatttctgacatactaagattttaacgactttcacaaatatgctgtactgagagagaatgttacataacattgagaactagtacaagtaaatattaaagtgaagtgaccatttcctacacaagctcattcagaggaggatgaagaccattttggaggaagaaaagcacccttattaagaattgcagcaagtaagccaacaaggtcttttcaggatgattttcttatatcaagtggtacatttcattttatttacttcagtttctggtgaatgtgtgactcagttgttgaaggacacctgctttgaaggaggggacattactacggtcttcacaccaagcgccaagtactgccaggtagtctgcacttaccacccaagatgtttactcttcactttcacggcggaatcaccatctgaggatcccacccgatggtttacttgtgtcctgaaagacagtgttacagaaacactgccaagagtgaataggacagcagcgatttctgggtattctttcaagcaatgctcacaccaaataagcgcttgcaacaaagacatttatgtggacctagacatgaagggcataaactataacagctcagttgccaagagtgctcaagaatgccaagaaagatgcacggatgacgtccactgccactttttcacgtacgccacaaggcagtttcccagcctggagcatcgtaacatttgtctactgaagcacacccaaacagggacaccaaccagaataacgaagctcgataaagtggtgtctggattttcactgaaatcctgtgcactttctaatctggcttgtattagggacattttccctaatacggtgtttgcagacagcaacatcgacagtgtcatggctcccgatgcttttgtctgtggccgaatctgcactcatcatcccggttgcttgttttttaccttcttttcccaggaatggcccaaagaatctcaaagaaatctttgtctccttaaaacatctgagagtggattgcccagtacacgcattaaaaagagcaaagctctttctggtttcagtctacaaagctgcaggcacagcatcccagtgttctgccattcttcattttaccatgacactgatttcttgggagaagaactggatattgttgctgcaaaaagtcacgaggcctgccagaaactgtgcaccaatgccgtccgctgccagttttttacctataccccagcccaagcatcctgcaacgaagggaagggcaagtgttacttaaagctttcttcaaacggatctccaactaaaatacttcacgggagaggaggcatctctggatacacattaaggttgtgtaaaatggataatgagtgtaccaccaaaatcaagcccaggatcgttggaggaactgcgtctgttcgtggtgagtggccgtggcaggtgaccctgcacacaacctcacccactcagagacacctgtgtggaggctccatcattggaaaccagtggatattaacagccgctcactgtttctatggggtagagtcacctaagattttgcgtgtctacagtggcattttaaatcaatctgaaataaaagaggacacatctttctttggggttcaagaaataataatccatgatcagtataaaatggcagaaagcgggtatgatattgccttgttgaaactggaaaccacagtgaattacacagattctcaacgacccatatgcctgccttccaaaggagatagaaatgtaatatacactgattgctgggtgactggatgggggtacagaaaactaagagacaaaatacaaaatactctccagaaagccaagatacccttagtgaccaacgaagagtgccagaagagatacagaggacataaaataacccataagatgatctgtgccggctacagggaaggagggaaggacgcttgcaagggagattcgggaggccctctgtcctgcaaacacaatgaggtctggcatctggtaggcatcacgagctggggcgaaggctgtgctcaaagggagcggccaggtgtttacaccaacgtggtcgagtacgtggactggattctggagaaaactcaagcagtgtgaatgggttcccaggggccattggagtccctgaaggacccaggatttgctgggagagggtgttgagttcactgtgccagcatgcttcctccacagtaacacgctgaaggggcttggtgtttgtaagaaaatgctagaagaaaacaaactgtcacaagttgttatgtccaaaactcccgttctatgatcgttgtagtttgtttgagcattcagtctctttgtttttgatcacgcttctatggagtccaagaattaccataaggcaatatttctgaagattactatataggcagatatagcagaaaataaccaagtagtggcagtggggatcaggcagaagaactggtaaaagaagccaccataaatagatttgttcgatgaaagatgaaaactggaagaaaggagaacaaagacagtcttcaccattttgcaggaatctacactctgcctatgtgaacacatttcttttgtaaagaaagaaattgattgcatttaatggcagattttcagaatagtcaggaattcttgtcatttccattttaaaatatatattaaaaaaaatcagttcgagtagacacgagctaagagtgaatgtgaagataacagaatttctgtgtggaagaggattacaagcagcaatttacctggaagtgataccttaggggcaatcttgaagatacactttcctgaaaaatgatttgtgatggattgtatatttatttaaaatatcttgggaggggaggctgatggagatagggagcatgctcaaacctccctaagacaagctgctgctgtgactatgggctcccaaagagctagatcgtatatttatttgacaaaaatcaccatagactgcatccatactacagagaaaaaacaattagggcgcaaatggatagttacagtaaagtcttcagcaagcagctgcctgtattctaagcactgggattttctgtttcgtgcaaatatttatctcattattgttgtgatctagttcaataacctagaatttgaattgtcaccacatagctttcaatctgtgccaacaactatacaattcatcaagtgtg

SEQ ID NO: 3 - protein, 5 aa, Artificial Sequence
  source: /note="Description of Artificial Sequence: Synthetic peptide"
TAAMS

SEQ ID NO: 4 - protein, 17 aa, Artificial Sequence
  source: /note="Description of Artificial Sequence: Synthetic peptide"
GISGSGSSTYYADSVKG

SEQ ID NO: 5 - protein, 13 aa, Artificial Sequence
  source: /note="Description of Artificial Sequence: Synthetic peptide"
ELSYLYSGYYFDY

SEQ ID NO: 6 - protein, 7 aa, Artificial Sequence
  source: /note="Description of Artificial Sequence: Synthetic peptide"
GFTFSTA

SEQ ID NO: 7 - protein, 6 aa, Artificial Sequence
  source: /note="Description of Artificial Sequence: Synthetic peptide"
SGSGSS

SEQ ID NO: 8 - protein, 13 aa, Artificial Sequence
  source: /note="Description of Artificial Sequence: Synthetic peptide"
ELSYLYSGYYFDY

SEQ ID NO: 9 - protein, 122 aa, Artificial Sequence
  source: /note="Description of Artificial Sequence: Synthetic polypeptide"
QVQLLESGGGLVQPGGSLRLSCAASGFTFSTAAMSWVRQAPGKGLEWVSGISGSGSSTYYADSVKGRFTISRDNSKNTLYLQMNSLRAEDTAVYYCARELSYLYSGYYFDYWGQGTLVTVSS

SEQ ID NO: 10 - DNA, 366 bp, Artificial Sequence
  source: /note="Description of Artificial Sequence: Synthetic polynucleotide"
caggtgcaattgctggaaagcggcggtggcctggtgcagccgggtggcagcctgcgtctgagctgcgcggcgtccggattcaccttttctactgctgctatgtcttgggtgcgccaggccccgggcaaaggtctcgagtgggtttccggtatctctggttctggttcttctacctactatgcggatagcgtgaaaggccgctttaccatcagccgcgataattcgaaaaacaccctgtatctgcaaatgaacagcctgcgtgcggaagatacggccgtgtattattgcgcgcgtgaactgtcttacctgtactctggttactacttcgattactggggccaaggcaccctggtgactgttagctca

SEQ ID NO: 11 - protein, 452 aa, Artificial Sequence
  source: /note="Description of Artificial Sequence: Synthetic polypeptide"
QVQLLESGGGLVQPGGSLRLSCAASGFTFSTAAMSWVRQAPGKGLEWVSGISGSGSSTYYADSVKGRFTISRDNSKNTLYLQMNSLRAEDTAVYYCARELSYLYSGYYFDYWGQGTLVTVSSASTKGPSVFPLAPSSKSTSGGTAALGCLVKDYFPEPVTVSWNSGALTSGVHTFPAVLQSSGLYSLSSVVTVPSSSLGTQTYICNVNHKPSNTKVDKRVEPKSCDKTHTCPPCPAPEAAGGPSVFLFPPKPKDTLMISRTPEVTCVVVDVSHEDPEVKFNWYVDGVEVHNAKTKPREEQYNSTYRVVSVLTVLHQDWLNGKEYKCKVSNKALPAPIEKTISKAKGQPREPQVYTLPPSREEMTKNQVSLTCLVKGFYPSDIAVEWESNGQPENNYKTTPPVLDSDGSFFLYSKLTVDKSRWQQGNVFSCSVMHEALHNHYTQKSLSLSPGK

SEQ ID NO: 12 - DNA, 1356 bp, Artificial Sequence
  source: /note="Description of Artificial Sequence: Synthetic polynucleotide"
caggtgcaattgctggaaagcggcggtggcctggtgcagccgggtggcagcctgcgtctgagctgcgcggcgtccggattcaccttttctactgctgctatgtcttgggtgcgccaggccccgggcaaaggtctcgagtgggtttccggtatctctggttctggttcttctacctactatgcggatagcgtgaaaggccgctttaccatcagccgcgataattcgaaaaacaccctgtatctgcaaatgaacagcctgcgtgcggaagatacggccgtgtattattgcgcgcgtgaactgtcttacctgtactctggttactacttcgattactggggccaaggcaccctggtgactgttagctcagcctccaccaagggtccatcggtcttccccctggcaccctcctccaagagcacctctgggggcacagcggccctgggctgcctggtcaaggactacttccccgaaccggtgacggtgtcgtggaactcaggcgccctgaccagcggcgtgcacaccttcccggctgtcctacagtcctcaggactctactccctcagcagcgtggtgaccgtgccctccagcagcttgggcacccagacctacatctgcaacgtgaatcacaagcccagcaacaccaaggtggacaagagagttgagcccaaatcttgtgacaaaactcacacatgcccaccgtgcccagcacctgaagcagcggggggaccgtcagtcttcctcttccccccaaaacccaaggacaccctcatgatctcccggacccctgaggtcacatgcgtggtggtggacgtgagccacgaagaccctgaggtcaagttcaactggtacgtggacggcgtggaggtgcataatgccaagacaaagccgcgggaggagcagtacaacagcacgtaccgggtggtcagcgtcctcaccgtcctgcaccaggactggctgaatggcaaggagtacaagtgcaaggtctccaacaaagccctcccagcccccatcgagaaaaccatctccaaagccaaagggcagccccgagaaccacaggtgtacaccctgcccccatcccgggaggagatgaccaagaaccaggtcagcctgacctgcctggtcaaaggcttctatcccagcgacatcgccgtggagtgggagagcaatgggcagccggagaacaactacaagaccacgcctcccgtgctggactccgacggctccttcttcctctacagcaagctcaccgtggacaagagcaggtggcagcaggggaacgtcttctcatgctccgtgatgcatgaggctctgcacaaccactacacgcagaagagcctctccctgtctccgggtaaa

SEQ ID NO: 13 - protein, 13 aa, Artificial Sequence
  source: /note="Description of Artificial Sequence: Synthetic peptide"
SGSSSNIGSNDVS

SEQ ID NO: 14 - protein, 7 aa, Artificial Sequence
  source: /note="Description of Artificial Sequence: Synthetic peptide"
KNYNRPS

SEQ ID NO: 15 - protein, 11 aa, Artificial Sequence
  source: /note="Description of Artificial Sequence: Synthetic peptide"
SAWDQRQFDVV

SEQ ID NO: 16 - protein, 9 aa, Artificial Sequence
  source: /note="Description of Artificial Sequence: Synthetic peptide"
SSSNIGSND

SEQ ID NO: 17 - protein, 3 aa, Artificial Sequence
  source: /note="Description of Artificial Sequence: Synthetic peptide"
KNY

SEQ ID NO: 18 - protein, 8 aa, Artificial Sequence
  source: /note="Description of Artificial Sequence: Synthetic peptide"
WDQRQFDV

SEQ ID NO: 19 - protein, 110 aa, Artificial Sequence
  source: /note="Description of Artificial Sequence: Synthetic polypeptide"
DIVLTQPPSVSGAPGQRVTISCSGSSSNIGSNDVSWYQQLPGTAPKLLIYKNYNRPSGVPDRFSGSKSGTSASLAITGLQAEDEADYYCSAWDQRQFDVVFGGGTKLTVL

SEQ ID NO: 20 - DNA, 330 bp, Artificial Sequence
  source: /note="Description of Artificial Sequence: Synthetic polynucleotide"
gatatcgtgctgacccagccgccgagcgtgagcggtgcaccgggccagcgcgtgaccattagctgtagcggcagcagcagcaacattggttctaacgacgtgtcttggtaccagcagctgccgggcacggcgccgaaactgctgatctacaaaaactacaaccgcccgagcggcgtgccggatcgctttagcggatccaaaagcggcaccagcgccagcctggcgattaccggcctgcaagcagaagacgaagcggattattactgctctgcttgggaccagcgtcagttcgacgttgtgtttggcggcggcacgaagttaaccgtccta

SEQ ID NO: 21 - protein, 216 aa, Artificial Sequence
  source: /note="Description of Artificial Sequence: Synthetic polypeptide"
DIVLTQPPSVSGAPGQRVTISCSGSSSNIGSNDVSWYQQLPGTAPKLLIYKNYNRPSGVPDRFSGSKSGTSASLAITGLQAEDEADYYCSAWDQRQFDVVFGGGTKLTVLGQPKAAPSVTLFPPSSEELQANKATLVCLISDFYPGAVTVAWKADSSPVKAGVETTTPSKQSNNKYAASSYLSLTPEQWKSHRSYSCQVTHEGSTVEKTVAPTECS

SEQ ID NO: 22 - DNA, 648 bp, Artificial Sequence
  source: /note="Description of Artificial Sequence: Synthetic polynucleotide"
gatatcgtgctgacccagccgccgagcgtgagcggtgcaccgggccagcgcgtgaccattagctgtagcggcagcagcagcaacattggttctaacgacgtgtcttggtaccagcagctgccgggcacggcgccgaaactgctgatctacaaaaactacaaccgcccgagcggcgtgccggatcgctttagcggatccaaaagcggcaccagcgccagcctggcgattaccggcctgcaagcagaagacgaagcggattattactgctctgcttgggaccagcgtcagttcgacgttgtgtttggcggcggcacgaagttaaccgtcctaggtcagcccaaggctgccccctcggtcactctgttcccgccctcctctgaggagcttcaagccaacaaggccacactggtgtgtctcataagtgacttctacccgggagccgtgacagtggcctggaaggcagatagcagccccgtcaaggcgggagtggagaccaccacaccctccaaacaaagcaacaacaagtacgcggccagcagctatctgagcctgacgcctgagcagtggaagtcccacagaagctacagctgccaggtcacgcatgaagggagcaccgtggagaagacagtggcccctacagaatgttca

SEQ ID NO: 23 - protein, 5 aa, Artificial Sequence
  source: /note="Description of Artificial Sequence: Synthetic peptide"
TAAMS

SEQ ID NO: 24 - protein, 17 aa, Artificial Sequence
  source: /note="Description of Artificial Sequence: Synthetic peptide"
GISGSGSSTYYADSVKG

SEQ ID NO: 25 - protein, 13 aa, Artificial Sequence
  source: /note="Description of Artificial Sequence: Synthetic peptide"
ELSYLYSGYYFDY

SEQ ID NO: 26 - protein, 7 aa, Artificial Sequence
  source: /note="Description of Artificial Sequence: Synthetic peptide"
GFTFSTA

SEQ ID NO: 27 - protein, 6 aa, Artificial Sequence
  source: /note="Description of Artificial Sequence: Synthetic peptide"
SGSGSS

SEQ ID NO: 28 - protein, 13 aa, Artificial Sequence
  source: /note="Description of Artificial Sequence: Synthetic peptide"
ELSYLYSGYYFDY

SEQ ID NO: 29 - protein, 122 aa, Artificial Sequence; identical to SEQ ID NO: 9
  source: /note="Description of Artificial Sequence: Synthetic polypeptide"

SEQ ID NO: 30 - DNA, 366 bp, Artificial Sequence
  source: /note="Description of Artificial Sequence: Synthetic polynucleotide"
caggtgcagctgctggaatcaggcggcggactggtgcagcctggcggtagcctgagactgagctgcgctgctagtggcttcacctttagcaccgccgctatgagctgggttcgacaggccccagggaaaggcctcgagtgggtctcagggattagcggtagcggctctagcacctactacgccgatagcgtgaagggccggttcactatctctagggataactctaagaacaccctgtacctgcagatgaatagcctgagagccgaggacaccgccgtctactactgcgctagagagctgagctacctgtatagcggctactacttcgactactggggtcaaggcaccctggtcaccgtgtctagc

SEQ ID NO: 31 - protein, 452 aa, Artificial Sequence
  source: /note="Description of Artificial Sequence: Synthetic polypeptide"
QVQLLESGGGLVQPGGSLRLSCAASGFTFSTAAMSWVRQAPGKGLEWVSGISGSGSSTYYADSVKGRFTISRDNSKNTLYLQMNSLRAEDTAVYYCARELSYLYSGYYFDYWGQGTLVTVSSASTKGPSVFPLAPSSKSTSGGTAALGCLVKDYFPEPVTVSWNSGALTSGVHTFPAVLQSSGLYSLSSVVTVPSSSLGTQTYICNVNHKPSNTKVDKRVEPKSCDKTHTCPPCPAPELLGGPSVFLFPPKPKDTLMISRTPEVTCVVVAVSHEDPEVKFNWYVDGVEVHNAKTKPREEQYNSTYRVVSVLTVLHQDWLNGKEYKCKVSNKALAAPIEKTISKAKGQPREPQVYTLPPSREEMTKNQVSLTCLVKGFYPSDIAVEWESNGQPENNYKTTPPVLDSDGSFFLYSKLTVDKSRWQQGNVFSCSVMHEALHNHYTQKSLSLSPGK

SEQ ID NO: 32 - DNA, 1356 bp, Artificial Sequence
  source: /note="Description of Artificial Sequence: Synthetic polynucleotide"
caggtgcagctgctggaatcaggcggcggactggtgcagcctggcggtagcctgagactgagctgcgctgctagtggcttcacctttagcaccgccgctatgagctgggttcgacaggccccagggaaaggcctcgagtgggtctcagggattagcggtagcggctctagcacctactacgccgatagcgtgaagggccggttcactatctctagggataactctaagaacaccctgtacctgcagatgaatagcctgagagccgaggacaccgccgtctactactgcgctagagagctgagctacctgtatagcggctactacttcgactactggggtcaaggcaccctggtcaccgtgtctagcgctagcactaagggcccctccgtgttccctctggccccttccagcaagtctacctccggcggcacagctgctctgggctgcctggtcaaggactacttccctgagcctgtgacagtgtcctggaactctggcgccctgacctctggcgtgcacaccttccctgccgtgctgcagtcctccggcctgtactccctgtcctccgtggtcacagtgccttcaagcagcctgggcacccagacctatatctgcaacgtgaaccacaagccttccaacaccaaggtggacaagcgggtggagcctaagtcctgcgacaagacccacacctgtcctccctgccctgctcctgaactgctgggcggcccttctgtgttcctgttccctccaaagcccaaggacaccctgatgatctcccggacccctgaagtgacctgcgtggtggtggccgtgtcccacgaggatcctgaagtgaagttcaattggtacgtggacggcgtggaggtgcacaacgccaagaccaagcctcgggaggaacagtacaactccacctaccgggtggtgtccgtgctgaccgtgctgcaccaggactggctgaacggcaaagagtacaagtgcaaagtctccaacaaggccctggccgcccctatcgaaaagacaatctccaaggccaagggccagcctagggaaccccaggtgtacaccctgccacccagccgggaggaaatgaccaagaaccaggtgtccctgacctgtctggtcaagggcttctacccttccgatatcgccgtggagtgggagtctaacggccagcctgagaacaactacaagaccacccctcctgtgctggactccgacggctccttcttcctgtactccaaactgaccgtggacaagtcccggtggcagcagggcaacgtgttctcctgctccgtgatgcacgaggccctgcacaaccactacacccagaagtccctgtccctgtctcccggcaag

SEQ ID NO: 33 - protein, 13 aa, Artificial Sequence
  source: /note="Description of Artificial Sequence: Synthetic peptide"
SGSSSNIGSNDVS

SEQ ID NO: 34 - protein, 7 aa, Artificial Sequence
  source: /note="Description of Artificial Sequence: Synthetic peptide"
KNYNRPS

SEQ ID NO: 35 - protein, 11 aa, Artificial Sequence
  source: /note="Description of Artificial Sequence: Synthetic peptide"
SAWDQRQFDVV

SEQ ID NO: 36 - protein, 9 aa, Artificial Sequence
  source: /note="Description of Artificial Sequence: Synthetic peptide"
SSSNIGSND

SEQ ID NO: 37 - protein, 3 aa, Artificial Sequence
  source: /note="Description of Artificial Sequence: Synthetic peptide"
KNY

SEQ ID NO: 38 - protein, 8 aa, Artificial Sequence
  source: /note="Description of Artificial Sequence: Synthetic peptide"
WDQRQFDV

SEQ ID NO: 39 - protein, 110 aa, Artificial Sequence
  source: /note="Description of Artificial Sequence: Synthetic polypeptide"
QSVLTQPPSASGTPGQRVTISCSGSSSNIGSNDVSWYQQLPGTAPKLLIYKNYNRPSGVPDRFSGSKSGTSASLAISGLQSEDEADYYCSAWDQRQFDVVFGGGTKLTVL

SEQ ID NO: 40 - DNA, 330 bp, Artificial Sequence
  source: /note="Description of Artificial Sequence: Synthetic polynucleotide"
cagtcagtcctgactcagccccctagcgctagtggcacccctggtcaaagagtgactattagctgtagcggctctagctctaatatcggctctaacgacgtcagctggtatcagcagctgcccggcaccgcccctaagctgctgatctataagaactataataggcctagcggcgtgcccgataggtttagcggatctaaatcagggacttctgctagtctggctattagcggcctgcagtcagaggacgaggccgactactactgtagcgcctgggatcagcgtcagttcgacgtggtgttcggcggaggcactaagctgaccgtgctg

SEQ ID NO: 41 - protein, 216 aa, Artificial Sequence
  source: /note="Description of Artificial Sequence: Synthetic polypeptide"
QSVLTQPPSASGTPGQRVTISCSGSSSNIGSNDVSWYQQLPGTAPKLLIYKNYNRPSGVPDRFSGSKSGTSASLAISGLQSEDEADYYCSAWDQRQFDVVFGGGTKLTVLGQPKAAPSVTLFPPSSEELQANKATLVCLISDFYPGAVTVAWKADSSPVKAGVETTTPSKQSNNKYAASSYLSLTPEQWKSHRSYSCQVTHEGSTVEKTVAPTECS

SEQ ID NO: 42 - DNA, 648 bp, Artificial Sequence
  source: /note="Description of Artificial Sequence: Synthetic polynucleotide"
cagtcagtcctgactcagccccctagcgctagtggcacccctggtcaaagagtgactattagctgtagcggctctagctctaatatcggctctaacgacgtcagctggtatcagcagctgcccggcaccgcccctaagctgctgatctataagaactataataggcctagcggcgtgcccgataggtttagcggatctaaatcagggacttctgctagtctggctattagcggcctgcagtcagaggacgaggccgactactactgtagcgcctgggatcagcgtcagttcgacgtggtgttcggcggaggcactaagctgaccgtgctgggtcaacctaaggctgcccccagcgtgaccctgttcccccccagcagcgaggagctgcaggccaacaaggccaccctggtgtgcctgatcagcgacttctacccaggcgccgtgaccgtggcctggaaggccgacagcagccccgtgaaggccggcgtggagaccaccacccccagcaagcagagcaacaacaagtacgccgccagcagctacctgagcctgacccccgagcagtggaagagccacaggtcctacagctgccaggtgacccacgagggcagcaccgtggaaaagaccgtggccccaaccgagtgcagc

SEQ ID NO: 43 - protein, 8 aa, Artificial Sequence
  source: /note="Description of Artificial Sequence: Synthetic peptide"
GFTFSTAA

SEQ ID NO: 44 - protein, 8 aa, Artificial Sequence
  source: /note="Description of Artificial Sequence: Synthetic peptide"
ISGSGSST

SEQ ID NO: 45 - protein, 15 aa, Artificial Sequence
  source: /note="Description of Artificial Sequence: Synthetic peptide"
ARELSYLYSGYYFDY

SEQ ID NO: 46 - protein, 10 aa, Artificial Sequence
  source: /note="Description of Artificial Sequence: Synthetic peptide"
GFTFSTAAMS

SEQ ID NO: 47 - protein, 8 aa, Artificial Sequence
  source: /note="Description of Artificial Sequence: Synthetic peptide"
SSNIGSND

SEQ ID NO: 48 - protein, 6 aa, Artificial Sequence
  source: /note="Description of Artificial Sequence: Synthetic 6xHis tag"
HHHHHH

SEQ ID NO: 49 - protein, 4 aa, Artificial Sequence
  source: /note="Description of Artificial Sequence: Synthetic peptide"
MGSS

SEQ ID NO: 50 - protein, 8 aa, Artificial Sequence
  source: /note="Description of Artificial Sequence: Synthetic 8xHis tag"
HHHHHHHH

SEQ ID NO: 51 - protein, 238 aa, Artificial Sequence
  source: /note="Description of Artificial Sequence: Synthetic polypeptide"
IVGGTASVRGEWPWQVTLHTTSPTQRHLCGGSIIGNQWILTAAHCFYGVESPKILRVYSGILNQSEIKEDTSFFGVQEIIIHDQYKMAESGYDIALLKLETTVNYTDSQRPICLPSKGDRNVIYTDCWVTGWGYRKLRDKIQNTLQKAKIPLVTNEECQKRYRGHKITHKMICAGYREGGKDACKGDSGGPLSCKHNEVWHLVGITSWGEGCAQRERPGVYTNVVEYVDWILEKTQAV